European Patent Specification EP 3 725 318 B1, published July 2, 2025. Title: Compositions for treating joint or connective tissue disease comprising dextran or poloxamer. Applicant: LEE, ILHOON PARK, YOOSIN. The sequence listing filed with the application follows.

SEQUENCE LISTING (10 sequences)

SEQ ID NO: 1 - DNA, 19 bp, Artificial Sequence
  MMP-3 forward primer
tgggaagccagtggaaatg

SEQ ID NO: 2 - DNA, 21 bp, Artificial Sequence
  MMP-3 reverse primer
ccatgcaatgggtaggatgag

SEQ ID NO: 3 - DNA, 20 bp, Artificial Sequence
  MMP-13 forward primer
ctgacctgggatttccaaaa

SEQ ID NO: 4 - DNA, 20 bp, Artificial Sequence
  MMP-13 reverse primer
acacgtggttccctgagaag

SEQ ID NO: 5 - DNA, 26 bp, Artificial Sequence
  GAPDH forward primer
ctcaactacatggtctacatgttcca

SEQ ID NO: 6 - DNA, 22 bp, Artificial Sequence
  GAPDH reverse primer
cttcccattctcagccttgact

SEQ ID NO: 7 - DNA, 20 bp, Artificial Sequence
  IL-6 forward primer
tgatggatgcttccaaactg

SEQ ID NO: 8 - DNA, 20 bp, Artificial Sequence
  IL-6 reverse primer
gagcattggaagttggggta

SEQ ID NO: 9 - DNA, 21 bp, Artificial Sequence
  IL-10 forward primer
gttgccaagccttgtcagaaa

SEQ ID NO: 10 - DNA, 20 bp, Artificial Sequence
  IL-10 reverse primer
tttctgggccatggttctct